European Patent Application EP 4 790 070 A1, published August 12, 2026. Title: 항-CD24 항체 또는 이의 항원 결합 단편 및 이의 용도. Applicant: 재단법인 대구경북과학기술원. The sequence listing filed with the application follows.

SEQUENCE LISTING (21 sequences)

SEQ ID NO: 1 - protein, 8 aa, synthetic construct
GFTFSSYG

SEQ ID NO: 2 - protein, 8 aa, synthetic construct
GFTVSSNY

SEQ ID NO: 3 - protein, 8 aa, synthetic construct
MSGDGLAT

SEQ ID NO: 4 - protein, 7 aa, synthetic construct
IYSGGST

SEQ ID NO: 5 - protein, 21 aa, synthetic construct
CARDSSSWYGGYYYYYGMDVW

SEQ ID NO: 6 - protein, 12 aa, synthetic construct [sequence omitted]

SEQ ID NO: 7 - protein, 6 aa, synthetic construct
QGISSW

SEQ ID NO: 8 - protein, 9 aa, synthetic construct
SSDVGGYDH

SEQ ID NO: 9 - protein, 11 aa, synthetic construct [sequence omitted]

SEQ ID NO: 10 - protein, 12 aa, synthetic construct [sequence omitted]

SEQ ID NO: 11 - protein, 130 aa, synthetic construct
MAQVQLLESGGGVVQPGRSLRLSCAASGFTFSSYGMHWVRQAPGKGLEWVSGMSGDGLATYYADSVKGRFTISRDNSKNTLYLQMNSLRAEDTAVYYCARDSSSWYGGYYYYYGMDVWGQGTTVTVSSGS

SEQ ID NO: 12 - protein, 120 aa, synthetic construct
MAQVQLVQSGGGLIQPGGSLRLSCAASGFTVSSNYMSWVRQAPGKGLEWVSVIYSGGSTYYADSVKGRFTISRDNSKNTLYLQMNSLRAEDTAVYYCAREYGDYFDYWGQGTLVTVSSGS

SEQ ID NO: 13 - protein, 108 aa, synthetic construct
DIQMTQSPSSVSASVGDRVTITCRASQGISSWLAWYQQKPGKAPKLLIYAASSLQSGVPPRFSGSGSGTDFTLTISSLQPEDFATYYCQQSYSTPLTFGGGTKVEIKR

SEQ ID NO: 14 - protein, 111 aa, synthetic construct
QSALTQPASVSGSPGQSITISCTGTSSDVGGYDHVSWYQQHPGKAPKLMIYEVTKRPSGVSDRFSGSKSGNTASLTISGLQADDEADYYCSSYAGSNSVLFGGGTQLTVLG

SEQ ID NO: 15 - protein, 243 aa, synthetic construct
MAQVQLLESGGGVVQPGRSLRLSCAASGFTFSSYGMHWVRQAPGKGLEWVSGMSGDGLATYYADSVKGRFTISRDNSKNTLYLQMNSLRAEDTAVYYCARDSSSWYGGYYYYYGMDVWGQGTTVTVSSGSGGGGSDIQMTQSPSSVSASVGDRVTITCRASQGISSWLAWYQQKPGKAPKLLIYAASSLQSGVPPRFSGSGSGTDFTLTISSLQPEDFATYYCQQSYSTPLTFGGGTKVEIKR

SEQ ID NO: 16 - protein, 236 aa, synthetic construct
MAQVQLVQSGGGLIQPGGSLRLSCAASGFTVSSNYMSWVRQAPGKGLEWVSVIYSGGSTYYADSVKGRFTISRDNSKNTLYLQMNSLRAEDTAVYYCAREYGDYFDYWGQGTLVTVSSGSGGGGSQSALTQPASVSGSPGQSITISCTGTSSDVGGYDHVSWYQQHPGKAPKLMIYEVTKRPSGVSDRFSGSKSGNTASLTISGLQADDEADYYCSSYAGSNSVLFGGGTQLTVLG

SEQ ID NO: 17 - protein, 482 aa, synthetic construct
MAQVQLLESGGGVVQPGRSLRLSCAASGFTFSSYGMHWVRQAPGKGLEWVSGMSGDGLATYYADSVKGRFTISRDNSKNTLYLQMNSLRAEDTAVYYCARDSSSWYGGYYYYYGMDVWGQGTTVTVSSGSGGGGSDIQMTQSPSSVSASVGDRVTITCRASQGISSWLAWYQQKPGKAPKLLIYAASSLQSGVPPRFSGSGSGTDFTLTISSLQPEDFATYYCQQSYSTPLTFGGGTKVEIKRGLGGLASEPKSCDKTHTCPPCPAPELLGGPSVFLFPPKPKDTLMISRTPEVTCVVVDVSHEDPEVKFNWYVDGVEVHNAKTKPREEQYNSTYRVVSVLTVLHQDWLNGKEYKCKVSNKALPAPIEKTISKAKGQPREPQVYTLPPSREEMTKNQVSLTCLVKGFYPSDIAVEWESNGQPENNYKTTPPVLDSDGSFFLYSKLTVDKSRWQQGNVFSCSVMHEALHNHYTQKSLSLSPGK

SEQ ID NO: 18 - protein, 475 aa, synthetic construct
MAQVQLVQSGGGLIQPGGSLRLSCAASGFTVSSNYMSWVRQAPGKGLEWVSVIYSGGSTYYADSVKGRFTISRDNSKNTLYLQMNSLRAEDTAVYYCAREYGDYFDYWGQGTLVTVSSGSGGGGSQSALTQPASVSGSPGQSITISCTGTSSDVGGYDHVSWYQQHPGKAPKLMIYEVTKRPSGVSDRFSGSKSGNTASLTISGLQADDEADYYCSSYAGSNSVLFGGGTQLTVLGGLGGLASEPKSCDKTHTCPPCPAPELLGGPSVFLFPPKPKDTLMISRTPEVTCVVVDVSHEDPEVKFNWYVDGVEVHNAKTKPREEQYNSTYRVVSVLTVLHQDWLNGKEYKCKVSNKALPAPIEKTISKAKGQPREPQVYTLPPSREEMTKNQVSLTCLVKGFYPSDIAVEWESNGQPENNYKTTPPVLDSDGSFFLYSKLTVDKSRWQQGNVFSCSVMHEALHNHYTQKSLSLSPGK

SEQ ID NO: 19 - protein, 232 aa, synthetic construct
EPKSCDKTHTCPPCPAPELLGGPSVFLFPPKPKDTLMISRTPEVTCVVVDVSHEDPEVKFNWYVDGVEVHNAKTKPREEQYNSTYRVVSVLTVLHQDWLNGKEYKCKVSNKALPAPIEKTISKAKGQPREPQVYTLPPSREEMTKNQVSLTCLVKGFYPSDIAVEWESNGQPENNYKTTPPVLDSDGSFFLYSKLTVDKSRWQQGNVFSCSVMHEALHNHYTQKSLSLSPGK

SEQ ID NO: 20 - DNA, 729 bp, synthetic construct
  source 1..729: mol_type = other DNA
atggcacaggtgcagctgttggagtctgggggaggcgtggtccagcctgggaggtccctgagactctcctgtgcagcctctggattcaccttcagtagctatggcatgcactgggtccgccaggctccagggaaggggctggagtgggtctcaggcatgagtggagatggtcttgccacgtactacgcggactccgtgaagggccgattcaccatctccagagacaattccaagaacacgctgtatctgcaaatgaacagcctgagagccgaggacacggctgtgtattactgtgcgagagatagcagcagctggtacggaggttactactactactacggtatggacgtctggggccaagggaccacggtcaccgtctcctcaggcagcggcggtggcggatccgacatccagatgacccagtctccatcttccgtgtctgcatctgtaggagacagagtcaccatcacttgtcgggcgagtcagggtattagcagctggttagcctggtatcagcagaaaccagggaaagcccctaagctcctgatctatgctgcatccagtttgcaaagtggggtcccaccaaggttcagtggcagtggatctgggacagatttcactctcaccatcagcagtctgcaacctgaagattttgcaacttactactgtcaacagagttacagtaccccgctcactttcggcggagggaccaaggtggagatcaaacgt

SEQ ID NO: 21 - DNA, 708 bp, synthetic construct
  source 1..708: mol_type = other DNA
atggcacaggtacagctggtgcagtctggaggaggcttgatccagcctggggggtccctgagactctcctgtgcagcctctgggttcaccgtcagtagcaactacatgagctgggtccgccaggctccagggaaggggctggagtgggtctcagttatttatagcggtggtagcacatactacgcagactccgtgaagggccgattcaccatctccagagacaattccaagaacacgctgtatcttcaaatgaacagcctgagagctgaggacacggctgtgtattactgtgcgagagagtacggtgactactttgactactggggccagggcaccctggtcaccgtctcctcaggcagcggcggtggcggatcccagtctgccctgactcagcctgcctccgtgtctgggtctcctggacagtcgatcaccatctcctgcactggaaccagtagtgacgtcggtggttatgaccatgtctcctggtaccaacaacacccaggcaaagcccccaaattgatgatttatgaggtcactaaacggccctcaggggtttctgatcgcttctctggctccaagtctggcaacacggcctccctgaccatctctgggctccaggctgacgatgaggctgattattactgcagctcatatgcaggcagcaacagtgtacttttcggcggagggacccagctcaccgttttaggt